European Patent Application EP 4 613 756 A2, published September 10, 2025. Title: HYBRIDIZATION CHAIN REACTION METHODS FOR IN SITU MOLECULAR DETECTION. Applicant: PRESIDENT AND FELLOWS OF HARVARD COLLEGE. Application EP. The sequence listing filed with the application follows.

SEQUENCE LISTING (104 sequences)

SEQ ID NO: 1 - DNA, 48 bp, synthetic construct
  misc_feature 1..48: note = Description of Artificial Sequence: Synthetic probe
  source 1..48: mol_type = other DNA
ccgaccgaaaagtgtgactgtataaatattctcggtacgtaccccgcc

SEQ ID NO: 2 - DNA, 48 bp, synthetic construct
  misc_feature 1..48: note = Description of Artificial Sequence: Synthetic probe
  source 1..48: mol_type = other DNA
tcatcaggggacaaaatgcctataatgacctccgtgcgaggatttact

SEQ ID NO: 3 - DNA, 48 bp, synthetic construct
  misc_feature 1..48: note = Description of Artificial Sequence: Synthetic probe
  source 1..48: mol_type = other DNA
gtcgatgtgtccaaagtgactatttaaaacggtttgtcggcagcccac

SEQ ID NO: 4 - DNA, 48 bp, synthetic construct
  misc_feature 1..48: note = Description of Artificial Sequence: Synthetic probe
  source 1..48: mol_type = other DNA
gagcagtagaagcacacacatataaccattcatcgctccgtcgcctta

SEQ ID NO: 5 - DNA, 48 bp, synthetic construct
  misc_feature 1..48: note = Description of Artificial Sequence: Synthetic probe
  source 1..48: mol_type = other DNA
catgcccagaataaagcacttatggaaaagtcgttggcggggtttacg

SEQ ID NO: 6 - DNA, 48 bp, synthetic construct
  misc_feature 1..48: note = Description of Artificial Sequence: Synthetic probe
  source 1..48: mol_type = other DNA
gcgtcaaatcatcctgattctataaatattctcggtacgtaccccgcc

SEQ ID NO: 7 - DNA, 48 bp, synthetic construct
  misc_feature 1..48: note = Description of Artificial Sequence: Synthetic probe
  source 1..48: mol_type = other DNA
ttgccttgatgatatcggactataatgacctccgtgcgaggatttact

SEQ ID NO: 8 - DNA, 48 bp, synthetic construct
  misc_feature 1..48: note = Description of Artificial Sequence: Synthetic probe
  source 1..48: mol_type = other DNA
gttagattctgggcaatggatatttaaaacggtttgtcggcagcccac

SEQ ID NO: 9 - DNA, 48 bp, synthetic construct
  misc_feature 1..48: note = Description of Artificial Sequence: Synthetic probe
  source 1..48: mol_type = other DNA
acaggttcatgcggaaagtctataaccattcatcgctccgtcgcctta

SEQ ID NO: 10 - DNA, 48 bp, synthetic construct
  misc_feature 1..48: note = Description of Artificial Sequence: Synthetic probe
  source 1..48: mol_type = other DNA
ccgtcgaaatcagcattgtatatggaaaagtcgttggcggggtttacg

SEQ ID NO: 11 - DNA, 48 bp, synthetic construct
  misc_feature 1..48: note = Description of Artificial Sequence: Synthetic probe
  source 1..48: mol_type = other DNA
tgatgaatacgtcgcgcttgtataaatattctcggtacgtaccccgcc

SEQ ID NO: 12 - DNA, 48 bp, synthetic construct
  misc_feature 1..48: note = Description of Artificial Sequence: Synthetic probe
  source 1..48: mol_type = other DNA
acatgagcagattcatcacctataatgacctccgtgcgaggatttact

SEQ ID NO: 13 - DNA, 48 bp, synthetic construct
  misc_feature 1..48: note = Description of Artificial Sequence: Synthetic probe
  source 1..48: mol_type = other DNA
gtgaccaagttccaggaaactatttaaaacggtttgtcggcagcccac

SEQ ID NO: 14 - DNA, 48 bp, synthetic construct
  misc_feature 1..48: note = Description of Artificial Sequence: Synthetic probe
  source 1..48: mol_type = other DNA
accaattgttgatcacggtctataaccattcatcgctccgtcgcctta

SEQ ID NO: 15 - DNA, 48 bp, synthetic construct
  misc_feature 1..48: note = Description of Artificial Sequence: Synthetic probe
  source 1..48: mol_type = other DNA
accaataccgatactatggctatggaaaagtcgttggcggggtttacg

SEQ ID NO: 16 - DNA, 48 bp, synthetic construct
  misc_feature 1..48: note = Description of Artificial Sequence: Synthetic probe
  source 1..48: mol_type = other DNA
cttgttctcgaacgtctgactataaatattctcggtacgtaccccgcc

SEQ ID NO: 17 - DNA, 48 bp, synthetic construct
  misc_feature 1..48: note = Description of Artificial Sequence: Synthetic probe
  source 1..48: mol_type = other DNA
gagcatcgtttaggatacggtataatgacctccgtgcgaggatttact

SEQ ID NO: 18 - DNA, 48 bp, synthetic construct
  misc_feature 1..48: note = Description of Artificial Sequence: Synthetic probe
  source 1..48: mol_type = other DNA
ccatagcctttagattgttgtatttaaaacggtttgtcggcagcccac

SEQ ID NO: 19 - DNA, 48 bp, synthetic construct
  misc_feature 1..48: note = Description of Artificial Sequence: Synthetic probe
  source 1..48: mol_type = other DNA
aaagtggggaagagtgcgtttataaccattcatcgctccgtcgcctta

SEQ ID NO: 20 - DNA, 48 bp, synthetic construct
  misc_feature 1..48: note = Description of Artificial Sequence: Synthetic probe
  source 1..48: mol_type = other DNA
acccatagcgtggaaatagatatggaaaagtcgttggcggggtttacg

SEQ ID NO: 21 - DNA, 48 bp, synthetic construct
  misc_feature 1..48: note = Description of Artificial Sequence: Synthetic probe
  source 1..48: mol_type = other DNA
cgactccatagcctttataatataaatattctcggtacgtaccccgcc

SEQ ID NO: 22 - DNA, 48 bp, synthetic construct
  misc_feature 1..48: note = Description of Artificial Sequence: Synthetic probe
  source 1..48: mol_type = other DNA
tggcatgttctggaactcaatataatgacctccgtgcgaggatttact

SEQ ID NO: 23 - DNA, 48 bp, synthetic construct
  misc_feature 1..48: note = Description of Artificial Sequence: Synthetic probe
  source 1..48: mol_type = other DNA
cgttgctccagtcaaatttgtatttaaaacggtttgtcggcagcccac

SEQ ID NO: 24 - DNA, 48 bp, synthetic construct
  misc_feature 1..48: note = Description of Artificial Sequence: Synthetic probe
  source 1..48: mol_type = other DNA
gaaaccaaacgatcccactctataaccattcatcgctccgtcgcctta

SEQ ID NO: 25 - DNA, 48 bp, synthetic construct
  misc_feature 1..48: note = Description of Artificial Sequence: Synthetic probe
  source 1..48: mol_type = other DNA
ttgtctcaaactgtcgcgattatggaaaagtcgttggcggggtttacg

SEQ ID NO: 26 - DNA, 48 bp, synthetic construct
  misc_feature 1..48: note = Description of Artificial Sequence: Synthetic probe
  source 1..48: mol_type = other DNA
tgcacattccagatcatacgtataaatattctcggtacgtaccccgcc

SEQ ID NO: 27 - DNA, 48 bp, synthetic construct
  misc_feature 1..48: note = Description of Artificial Sequence: Synthetic probe
  source 1..48: mol_type = other DNA
ggattaggcactggaatagctataatgacctccgtgcgaggatttact

SEQ ID NO: 28 - DNA, 48 bp, synthetic construct
  misc_feature 1..48: note = Description of Artificial Sequence: Synthetic probe
  source 1..48: mol_type = other DNA
gaaacgcgtctcgatttctctatttaaaacggtttgtcggcagcccac

SEQ ID NO: 29 - DNA, 48 bp, synthetic construct
  misc_feature 1..48: note = Description of Artificial Sequence: Synthetic probe
  source 1..48: mol_type = other DNA
acccaatgttacgttctttgtataaccattcatcgctccgtcgcctta

SEQ ID NO: 30 - DNA, 48 bp, synthetic construct
  misc_feature 1..48: note = Description of Artificial Sequence: Synthetic probe
  source 1..48: mol_type = other DNA
gggctttttggatatgttgatatggaaaagtcgttggcggggtttacg

SEQ ID NO: 31 - DNA, 48 bp, synthetic construct
  misc_feature 1..48: note = Description of Artificial Sequence: Synthetic probe
  source 1..48: mol_type = other DNA
gatcaaagtcgggcatttcgtataaatattctcggtacgtaccccgcc

SEQ ID NO: 32 - DNA, 48 bp, synthetic construct
  misc_feature 1..48: note = Description of Artificial Sequence: Synthetic probe
  source 1..48: mol_type = other DNA
tcaatacgtagcaaccagggtataatgacctccgtgcgaggatttact

SEQ ID NO: 33 - DNA, 48 bp, synthetic construct
  misc_feature 1..48: note = Description of Artificial Sequence: Synthetic probe
  source 1..48: mol_type = other DNA
ttgttctcttcgttgttcattatttaaaacggtttgtcggcagcccac

SEQ ID NO: 34 - DNA, 48 bp, synthetic construct
  misc_feature 1..48: note = Description of Artificial Sequence: Synthetic probe
  source 1..48: mol_type = other DNA
ctcaatgcagcgcaagaacatataaccattcatcgctccgtcgcctta

SEQ ID NO: 35 - DNA, 48 bp, synthetic construct
  misc_feature 1..48: note = Description of Artificial Sequence: Synthetic probe
  source 1..48: mol_type = other DNA
cagtgatcacgatacgcttctatggaaaagtcgttggcggggtttacg

SEQ ID NO: 36 - DNA, 48 bp, synthetic construct
  misc_feature 1..48: note = Description of Artificial Sequence: Synthetic probe
  source 1..48: mol_type = other DNA
cactttcatcatcgatgtgctataaatattctcggtacgtaccccgcc

SEQ ID NO: 37 - DNA, 48 bp, synthetic construct
  misc_feature 1..48: note = Description of Artificial Sequence: Synthetic probe
  source 1..48: mol_type = other DNA
gtcatcacatcgcacaacagtataatgacctccgtgcgaggatttact

SEQ ID NO: 38 - DNA, 48 bp, synthetic construct
  misc_feature 1..48: note = Description of Artificial Sequence: Synthetic probe
  source 1..48: mol_type = other DNA
cgtattgggaatctcgatgctatttaaaacggtttgtcggcagcccac

SEQ ID NO: 39 - DNA, 48 bp, synthetic construct
  misc_feature 1..48: note = Description of Artificial Sequence: Synthetic probe
  source 1..48: mol_type = other DNA
gagtatcccgatgaagatggtataaccattcatcgctccgtcgcctta

SEQ ID NO: 40 - DNA, 48 bp, synthetic construct
  misc_feature 1..48: note = Description of Artificial Sequence: Synthetic probe
  source 1..48: mol_type = other DNA
caaacgacggactcgactggtatggaaaagtcgttggcggggtttacg

SEQ ID NO: 41 - DNA, 48 bp, synthetic construct
  misc_feature 1..48: note = Description of Artificial Sequence: Synthetic probe
  source 1..48: mol_type = other DNA
aattgggggagtagttggactataaatattctcggtacgtaccccgcc

SEQ ID NO: 42 - DNA, 48 bp, synthetic construct
  misc_feature 1..48: note = Description of Artificial Sequence: Synthetic probe
  source 1..48: mol_type = other DNA
cgatgtgggcgaatagcaagtataatgacctccgtgcgaggatttact

SEQ ID NO: 43 - DNA, 48 bp, synthetic construct
  misc_feature 1..48: note = Description of Artificial Sequence: Synthetic probe
  source 1..48: mol_type = other DNA
gctgaatagttcggacttgttatttaaaacggtttgtcggcagcccac

SEQ ID NO: 44 - DNA, 48 bp, synthetic construct
  misc_feature 1..48: note = Description of Artificial Sequence: Synthetic probe
  source 1..48: mol_type = other DNA
tggcgtatattgtggtgatctataaccattcatcgctccgtcgcctta

SEQ ID NO: 45 - DNA, 48 bp, synthetic construct
  misc_feature 1..48: note = Description of Artificial Sequence: Synthetic probe
  source 1..48: mol_type = other DNA
gcgagtagatggacatgttctatggaaaagtcgttggcggggtttacg

SEQ ID NO: 46 - DNA, 48 bp, synthetic construct
  misc_feature 1..48: note = Description of Artificial Sequence: Synthetic probe
  source 1..48: mol_type = other DNA
gcgtagtcggtacttaactatataaatattctcggtacgtaccccgcc

SEQ ID NO: 47 - DNA, 48 bp, synthetic construct
  misc_feature 1..48: note = Description of Artificial Sequence: Synthetic probe
  source 1..48: mol_type = other DNA
cttcgaattcgcttttctggtataatgacctccgtgcgaggatttact

SEQ ID NO: 48 - DNA, 48 bp, synthetic construct
  misc_feature 1..48: note = Description of Artificial Sequence: Synthetic probe
  source 1..48: mol_type = other DNA
acatttgtgtgcaggcgaaatatttaaaacggtttgtcggcagcccac

SEQ ID NO: 49 - DNA, 66 bp, synthetic construct
  misc_feature 1..66: note = Description of Artificial Sequence: Synthetic oligonucleotide
  modified_base 39: mod_base = OTHER; note = 5'Thiol-d-Inosine
  source 1..66: mol_type = other DNA
gaggagggcagcaaacgggaagagtcttcctttacgttnttggcggggtacgtaccgagaatattt

SEQ ID NO: 50 - DNA, 66 bp, synthetic construct
  misc_feature 1..66: note = Description of Artificial Sequence: Synthetic oligonucleotide
  modified_base 39: mod_base = OTHER; note = 5'Thiol-d-Inosine
  source 1..66: mol_type = other DNA
cctcgtaaatcctcatcaatcatccagtaaaccgccttntttaacacgggaaacactacggacatt

SEQ ID NO: 51 - DNA, 66 bp, synthetic construct
  misc_feature 1..66: note = Description of Artificial Sequence: Synthetic oligonucleotide
  modified_base 39: mod_base = OTHER; note = 5'Thiol-d-Inosine
  source 1..66: mol_type = other DNA
gtccctgcctctatatctccactcaactttaacccgttnttatgctaacatccggggtcaccgtac

SEQ ID NO: 52 - DNA, 66 bp, synthetic construct
  misc_feature 1..66: note = Description of Artificial Sequence: Synthetic oligonucleotide
  modified_base 39: mod_base = OTHER; note = 5'Thiol-d-Inosine
  source 1..66: mol_type = other DNA
cctcaacctacctccaactctcaccatattcgcttcttntttaggcgatccgtcgtatactgtacc

SEQ ID NO: 53 - DNA, 66 bp, synthetic construct
  misc_feature 1..66: note = Description of Artificial Sequence: Synthetic oligonucleotide
  modified_base 39: mod_base = OTHER; note = 5'Thiol-d-Inosine
  source 1..66: mol_type = other DNA
gaggagggcagcaaacgggaagagtcttcctttacgttnttagtaaatcctcgcacggaggtcatt

SEQ ID NO: 54 - DNA, 66 bp, synthetic construct
  misc_feature 1..66: note = Description of Artificial Sequence: Synthetic oligonucleotide
  modified_base 39: mod_base = OTHER; note = 5'Thiol-d-Inosine
  source 1..66: mol_type = other DNA
cctcgtaaatcctcatcaatcatccagtaaaccgccttntttgcgttacgagatagctcggacctt

SEQ ID NO: 55 - DNA, 66 bp, synthetic construct
  misc_feature 1..66: note = Description of Artificial Sequence: Synthetic oligonucleotide
  modified_base 39: mod_base = OTHER; note = 5'Thiol-d-Inosine
  source 1..66: mol_type = other DNA
gtccctgcctctatatctccactcaactttaacccgttnttgatctctgtccgacgcacaaccgtt

SEQ ID NO: 56 - DNA, 66 bp, synthetic construct
  misc_feature 1..66: note = Description of Artificial Sequence: Synthetic oligonucleotide
  modified_base 39: mod_base = OTHER; note = 5'Thiol-d-Inosine
  source 1..66: mol_type = other DNA
cctcaacctacctccaactctcaccatattcgcttcttnttgcgcgttgggtaacttcgacgtcaa

SEQ ID NO: 57 - DNA, 66 bp, synthetic construct
  misc_feature 1..66: note = Description of Artificial Sequence: Synthetic oligonucleotide
  modified_base 39: mod_base = OTHER; note = 5'Thiol-d-Inosine
  source 1..66: mol_type = other DNA
gaggagggcagcaaacgggaagagtcttcctttacgttnttgtgggctgccgacaaaccgttttaa

SEQ ID NO: 58 - DNA, 66 bp, synthetic construct
  misc_feature 1..66: note = Description of Artificial Sequence: Synthetic oligonucleotide
  modified_base 39: mod_base = OTHER; note = 5'Thiol-d-Inosine
  source 1..66: mol_type = other DNA
cctcgtaaatcctcatcaatcatccagtaaaccgccttnttattgtccgcccggtaaatcaatgaa

SEQ ID NO: 59 - DNA, 66 bp, synthetic construct
  misc_feature 1..66: note = Description of Artificial Sequence: Synthetic oligonucleotide
  modified_base 39: mod_base = OTHER; note = 5'Thiol-d-Inosine
  source 1..66: mol_type = other DNA
gtccctgcctctatatctccactcaactttaacccgttnttggactccgcacgttcgagaacactt

SEQ ID NO: 60 - DNA, 66 bp, synthetic construct
  misc_feature 1..66: note = Description of Artificial Sequence: Synthetic oligonucleotide
  modified_base 39: mod_base = OTHER; note = 5'Thiol-d-Inosine
  source 1..66: mol_type = other DNA
cctcaacctacctccaactctcaccatattcgcttcttnttttaattcactccacgcgaacgcgaa

SEQ ID NO: 61 - DNA, 66 bp, synthetic construct
  misc_feature 1..66: note = Description of Artificial Sequence: Synthetic oligonucleotide
  modified_base 39: mod_base = OTHER; note = 5'Thiol-d-Inosine
  source 1..66: mol_type = other DNA
gaggagggcagcaaacgggaagagtcttcctttacgttntttaaggcgacggagcgatgaatggtt

SEQ ID NO: 62 - DNA, 66 bp, synthetic construct
  misc_feature 1..66: note = Description of Artificial Sequence: Synthetic oligonucleotide
  modified_base 39: mod_base = OTHER; note = 5'Thiol-d-Inosine
  source 1..66: mol_type = other DNA
cctcgtaaatcctcatcaatcatccagtaaaccgccttnttccacaggtcaagttcgttagaacca

SEQ ID NO: 63 - DNA, 66 bp, synthetic construct
  misc_feature 1..66: note = Description of Artificial Sequence: Synthetic oligonucleotide
  modified_base 39: mod_base = OTHER; note = 5'Thiol-d-Inosine
  source 1..66: mol_type = other DNA
gtccctgcctctatatctccactcaactttaacccgttnttggactacgtcgtaagtctaaccctt

SEQ ID NO: 64 - DNA, 66 bp, synthetic construct
  misc_feature 1..66: note = Description of Artificial Sequence: Synthetic oligonucleotide
  modified_base 39: mod_base = OTHER; note = 5'Thiol-d-Inosine
  source 1..66: mol_type = other DNA
cctcaacctacctccaactctcaccatattcgcttcttntttttcgtgcgcaatcgactgtgggaa

SEQ ID NO: 65 - DNA, 66 bp, synthetic construct
  misc_feature 1..66: note = Description of Artificial Sequence: Synthetic oligonucleotide
  modified_base 39: mod_base = OTHER; note = 5'Thiol-d-Inosine
  source 1..66: mol_type = other DNA
gaggagggcagcaaacgggaagagtcttcctttacgttnttcgtaaaccccgccaacgacttttcc

SEQ ID NO: 66 - DNA, 66 bp, synthetic construct
  misc_feature 1..66: note = Description of Artificial Sequence: Synthetic oligonucleotide
  modified_base 39: mod_base = OTHER; note = 5'Thiol-d-Inosine
  source 1..66: mol_type = other DNA
cctcgtaaatcctcatcaatcatccagtaaaccgccttnttttggtgggactccgacctacaacaa

SEQ ID NO: 67 - DNA, 66 bp, synthetic construct
  misc_feature 1..66: note = Description of Artificial Sequence: Synthetic oligonucleotide
  modified_base 39: mod_base = OTHER; note = 5'Thiol-d-Inosine
  source 1..66: mol_type = other DNA
gtccctgcctctatatctccactcaactttaacccgttnttccgctgtagtcgttagttggcagtt

SEQ ID NO: 68 - DNA, 66 bp, synthetic construct
  misc_feature 1..66: note = Description of Artificial Sequence: Synthetic oligonucleotide
  modified_base 39: mod_base = OTHER; note = 5'Thiol-d-Inosine
  source 1..66: mol_type = other DNA
cctcaacctacctccaactctcaccatattcgcttcttntttactaaggtagccggactagggtcc

SEQ ID NO: 69 - DNA, 36 bp, synthetic construct
  misc_feature 1..36: note = Description of Artificial Sequence: Synthetic oligonucleotide
  source 1..36: mol_type = other DNA
gaggagggcagcaaacgggaagagtcttcctttacg

SEQ ID NO: 70 - DNA, 36 bp, synthetic construct
  misc_feature 1..36: note = Description of Artificial Sequence: Synthetic oligonucleotide
  source 1..36: mol_type = other DNA
cctcgtaaatcctcatcaatcatccagtaaaccgcc

SEQ ID NO: 71 - DNA, 36 bp, synthetic construct
  misc_feature 1..36: note = Description of Artificial Sequence: Synthetic oligonucleotide
  source 1..36: mol_type = other DNA
gtccctgcctctatatctccactcaactttaacccg

SEQ ID NO: 72 - DNA, 36 bp, synthetic construct
  misc_feature 1..36: note = Description of Artificial Sequence: Synthetic oligonucleotide
  source 1..36: mol_type = other DNA
cctcaacctacctccaactctcaccatattcgcttc

SEQ ID NO: 73 - DNA, 72 bp, synthetic construct
  misc_feature 1..72: note = Description of Artificial Sequence: Synthetic oligonucleotide
  modified_base 37: mod_base = OTHER; note = 5'Thiol-d-Inosine
  source 1..72: mol_type = other DNA
cgtaaaggaagactcttcccgtttgctgccctcctcncattctttcttgaggagggcagcaaacgggaagag

SEQ ID NO: 74 - DNA, 72 bp, synthetic construct
  misc_feature 1..72: note = Description of Artificial Sequence: Synthetic oligonucleotide
  modified_base 37: mod_base = OTHER; note = 5'Thiol-d-Inosine
  source 1..72: mol_type = other DNA
gaggagggcagcaaacgggaagagtcttcctttacgntcttcccgtttgctgccctcctcaagaaagaatgc

SEQ ID NO: 75 - DNA, 72 bp, synthetic construct; identical to SEQ ID NO: 73
  misc_feature 1..72: note = Description of Artificial Sequence: Synthetic oligonucleotide
  modified_base 37: mod_base = OTHER; note = 5'Thiol-d-Inosine
  source 1..72: mol_type = other DNA

SEQ ID NO: 76 - DNA, 72 bp, synthetic construct; identical to SEQ ID NO: 74
  misc_feature 1..72: note = Description of Artificial Sequence: Synthetic oligonucleotide
  modified_base 37: mod_base = OTHER; note = 5'Thiol-d-Inosine
  source 1..72: mol_type = other DNA

SEQ ID NO: 77 - DNA, 72 bp, synthetic construct
  misc_feature 1..72: note = Description of Artificial Sequence: Synthetic oligonucleotide
  misc_feature 1..72: note = Description of Combined DNA/RNA Molecule: Synthetic oligonucleotide
  source 1..72: mol_type = other DNA
cgtaaaggaagactcttcccgtttgctgccctcctcgcattctttcttgaggagggcagcaaacgggaagag

SEQ ID NO: 78 - DNA, 72 bp, synthetic construct
  misc_feature 1..72: note = Description of Artificial Sequence: Synthetic oligonucleotide
  misc_feature 1..72: note = Description of Combined DNA/RNA Molecule: Synthetic oligonucleotide
  source 1..72: mol_type = other DNA
gaggagggcagcaaacgggaagagtcttcctttacgctcttcccgtttgctgccctcctcaagaaagaatgc

SEQ ID NO: 79 - DNA, 72 bp, synthetic construct
  misc_feature 1..72: note = Description of Artificial Sequence: Synthetic oligonucleotide
  modified_base 3: mod_base = i
  modified_base 14: mod_base = i
  modified_base 24: mod_base = i
  modified_base 35: mod_base = i
  modified_base 45: mod_base = i
  source 1..72: mol_type = other DNA
cgnaaaggaagacncttcccgttngctgccctccncgcattcttncttgaggagggcagcaaacgggaagag

SEQ ID NO: 80 - DNA, 72 bp, synthetic construct
  misc_feature 1..72: note = Description of Artificial Sequence: Synthetic oligonucleotide
  modified_base 25: mod_base = i
  modified_base 33: mod_base = i
  modified_base 47: mod_base = i
  modified_base 59: mod_base = i
  modified_base 70: mod_base = i
  source 1..72: mol_type = other DNA
gaggagggcagcaaacgggaagagncttccttnacgctcttcccgtntgctgccctccncaagaaagaangc

SEQ ID NO: 81 - DNA, 84 bp, synthetic construct
  misc_feature 1..84: note = Description of Artificial Sequence: Synthetic oligonucleotide
  source 1..84: mol_type = other DNA
cagtaaaccgcccgggttaaagttgagtggagatatagaggcagggacaaagtctaatccgtccctgcctctatatctccactc

SEQ ID NO: 82 - DNA, 92 bp, synthetic construct
  misc_feature 1..92: note = Description of Artificial Sequence: Synthetic oligonucleotide
  source 1..92: mol_type = other DNA
tcttcagcgttcccgagacacgtaaaggaagactcttcccgtttgctgccctcctcgcattctttcttgaggagggcagcaaacgggaagag

SEQ ID NO: 83 - DNA, 90 bp, synthetic construct
  misc_feature 1..90: note = Description of Artificial Sequence: Synthetic oligonucleotide
  source 1..90: mol_type = other DNA
gaggagggcagcaaacgggaagagtcttcctttacgctcttcccgtttgctgccctcctcaagaaagaatgctcttcagcgttcccgaga

SEQ ID NO: 84 - DNA, 19 bp, synthetic construct
  misc_feature 1..19: note = Description of Artificial Sequence: Synthetic probe
  modified_base 19: mod_base = OTHER; note = 5'Thiol-d-Inosine
  source 1..19: mol_type = other DNA
tctcgggaacgctgaagan

SEQ ID NO: 85 - DNA, 25 bp, synthetic construct
  misc_feature 1..25: note = Description of Artificial Sequence: Synthetic probe
  source 1..25: mol_type = other DNA
ggcggggtacgtaccgagaatattt

SEQ ID NO: 86 - DNA, 25 bp, synthetic construct
  misc_feature 1..25: note = Description of Artificial Sequence: Synthetic probe
  source 1..25: mol_type = other DNA
taacacgggaaacactacggacatt

SEQ ID NO: 87 - DNA, 25 bp, synthetic construct
  misc_feature 1..25: note = Description of Artificial Sequence: Synthetic probe
  source 1..25: mol_type = other DNA
atgctaacatccggggtcaccgtac

SEQ ID NO: 88 - DNA, 25 bp, synthetic construct
  misc_feature 1..25: note = Description of Artificial Sequence: Synthetic probe
  source 1..25: mol_type = other DNA
taggcgatccgtcgtatactgtacc

SEQ ID NO: 89 - DNA, 25 bp, synthetic construct
  misc_feature 1..25: note = Description of Artificial Sequence: Synthetic probe
  source 1..25: mol_type = other DNA
agtaaatcctcgcacggaggtcatt

SEQ ID NO: 90 - DNA, 25 bp, synthetic construct
  misc_feature 1..25: note = Description of Artificial Sequence: Synthetic probe
  source 1..25: mol_type = other DNA
tgcgttacgagatagctcggacctt

SEQ ID NO: 91 - DNA, 25 bp, synthetic construct
  misc_feature 1..25: note = Description of Artificial Sequence: Synthetic probe
  source 1..25: mol_type = other DNA
gatctctgtccgacgcacaaccgtt

SEQ ID NO: 92 - DNA, 25 bp, synthetic construct
  misc_feature 1..25: note = Description of Artificial Sequence: Synthetic probe
  source 1..25: mol_type = other DNA
gcgcgttgggtaacttcgacgtcaa

SEQ ID NO: 93 - DNA, 25 bp, synthetic construct
  misc_feature 1..25: note = Description of Artificial Sequence: Synthetic probe
  source 1..25: mol_type = other DNA
gtgggctgccgacaaaccgttttaa

SEQ ID NO: 94 - DNA, 25 bp, synthetic construct
  misc_feature 1..25: note = Description of Artificial Sequence: Synthetic probe
  source 1..25: mol_type = other DNA
attgtccgcccggtaaatcaatgaa

SEQ ID NO: 95 - DNA, 25 bp, synthetic construct
  misc_feature 1..25: note = Description of Artificial Sequence: Synthetic probe
  source 1..25: mol_type = other DNA
ggactccgcacgttcgagaacactt

SEQ ID NO: 96 - DNA, 25 bp, synthetic construct
  misc_feature 1..25: note = Description of Artificial Sequence: Synthetic probe
  source 1..25: mol_type = other DNA
ttaattcactccacgcgaacgcgaa

SEQ ID NO: 97 - DNA, 25 bp, synthetic construct
  misc_feature 1..25: note = Description of Artificial Sequence: Synthetic probe
  source 1..25: mol_type = other DNA
taaggcgacggagcgatgaatggtt

SEQ ID NO: 98 - DNA, 25 bp, synthetic construct
  misc_feature 1..25: note = Description of Artificial Sequence: Synthetic probe
  source 1..25: mol_type = other DNA
ccacaggtcaagttcgttagaacca

SEQ ID NO: 99 - DNA, 25 bp, synthetic construct
  misc_feature 1..25: note = Description of Artificial Sequence: Synthetic probe
  source 1..25: mol_type = other DNA
ggactacgtcgtaagtctaaccctt

SEQ ID NO: 100 - DNA, 25 bp, synthetic construct
  misc_feature 1..25: note = Description of Artificial Sequence: Synthetic probe
  source 1..25: mol_type = other DNA
tttcgtgcgcaatcgactgtgggaa

SEQ ID NO: 101 - DNA, 25 bp, synthetic construct
  misc_feature 1..25: note = Description of Artificial Sequence: Synthetic probe
  source 1..25: mol_type = other DNA
cgtaaaccccgccaacgacttttcc

SEQ ID NO: 102 - DNA, 25 bp, synthetic construct
  misc_feature 1..25: note = Description of Artificial Sequence: Synthetic probe
  source 1..25: mol_type = other DNA
ttggtgggactccgacctacaacaa

SEQ ID NO: 103 - DNA, 25 bp, synthetic construct
  misc_feature 1..25: note = Description of Artificial Sequence: Synthetic probe
  source 1..25: mol_type = other DNA
ccgctgtagtcgttagttggcagtt

SEQ ID NO: 104 - DNA, 25 bp, synthetic construct
  misc_feature 1..25: note = Description of Artificial Sequence: Synthetic probe
  source 1..25: mol_type = other DNA
tactaaggtagccggactagggtcc